European Patent Application EP 4 545 642 A1, published April 30, 2025. Title: PHENOLIC COMPOUND PRODUCTION METHOD, AND MODIFIED ENZYME. Applicant: Tokyo University of Science Foundation. Application JP PCT/JP2023/027278, filed July 25, 2023. The sequence listing filed with the application follows.

SEQUENCE LISTING (16 sequences)

SEQ ID NO: 1 - protein, 603 aa, Thermothelomyces thermophila
MAHIHDLAPEVSNYSSGRLTPPTPVRFPRTPVFASMNKPCRFEGDVFDLEVSGAIPPDIDGTFFRVQPDHRFPPLFEDDIHFNGDGSVTAIRISGGHADLRQRYVRTERYLLETRARRSLFGRYRNPWTDNESVRGVIRTASNTNVVFWRGALLAMKEDGPPFAMDPVTLETLGRYDFEGQILSPTFTAHPKIDPDTGEMVCFAYEAGGDGSDCSVDVAVWTVDADGKKVEECWYKAPFAGMIHDCGITKNWVVLPLTPIKMDLERMKRGGNKFAWDPSEDQWYGVVPRRGAKSDDIIWFRADNGFHGHVAGCYELPSGEIVFDLTVADGNVFFFFPPDDNITPPADGVAKRNRLSSPTVRWIFDPKAKKSAIRTEAAGDADIWVADERVKPALTWPTNGEFSRIDDRYVTKPYRHFWQAVVDPTRPYDFEKCGPPAGGLFNCLGHYTWSDQNYHHGHNTGDPSGDGRSNGSAEEATAGKFGLQDVYFAGPTMTFQEPTFIPRQGAAEGEGYLIALLNHLDELRNDVVIFEARNLGKGPLAVIHLPLKLKLGLHGNWVDSREIEAWRRRRAENGDVGPLRVAKEPLPWQKKFAAAAQNGSNGV

SEQ ID NO: 2 - protein, 603 aa, synthetic construct
MAHIHDLAPEVSNYSSGRLTPPTPVRFPRTPVFASMNKPCRFEGDVFDLEVSGAIPPDIDGTFFRVQPDHRFPPLFEDDIHYNGDGSVTAIRISGGHADLRQRYVRTERYLLETRARRSLFGRYRNPWTDNESVRGVIRTASNTNVVFWRGALLAMKEDGPPFAMDPVTLETLGRYDFEGQILSPTFTAHPKIDPDTGEMVCFAYEAGGDGSDCSVDVAVWTVDADGKKVEECWYKAPFAGMIHDCGITKNWVVLPLTPIKMDLERMKRGGNKFAWDPSEDQWYGVVPRRGAKSDDIIWFRADNGFHGHVAGCYELPSGEIVFDLTVADGNVFFFFPPDDNITPPADGVAKRNRLSSPTVRWIFDPKAKKSAIRTEAAGDADIWVADERVKPALTWPTNGEFSRIDDRYVTKPYRHFWQAVVDPTRPYDFEKCGPPAGGLFNCLGHYTWSDQNYHHGHNTGDPSGDGRSNGSAEEATAGKFGLQDVYFAGPTMTFQEPTFIPRQGAAEGEGYLIALLNHLDELRNDVVIFEARNLGKGPLAVIHLPLKLKLGLHGNWVDSREIEAWRRRRAENGDVGPLRVAKEPLPWQKKFAAAAQNGSNGV

SEQ ID NO: 3 - protein, 603 aa, synthetic construct
MAHIHDLAPEVSNYSSGRLTPPTPVRFPRTPVFASMNKPCRFEGDVFDLEVSGAIPPDIDGTFFRVQPDHRFPPLFEDDIHWNGDGSVTAIRISGGHADLRQRYVRTERYLLETRARRSLFGRYRNPWTDNESVRGVIRTASNTNVVFWRGALLAMKEDGPPFAMDPVTLETLGRYDFEGQILSPTFTAHPKIDPDTGEMVCFAYEAGGDGSDCSVDVAVWTVDADGKKVEECWYKAPFAGMIHDCGITKNWVVLPLTPIKMDLERMKRGGNKFAWDPSEDQWYGVVPRRGAKSDDIIWFRADNGFHGHVAGCYELPSGEIVFDLTVADGNVFFFFPPDDNITPPADGVAKRNRLSSPTVRWIFDPKAKKSAIRTEAAGDADIWVADERVKPALTWPTNGEFSRIDDRYVTKPYRHFWQAVVDPTRPYDFEKCGPPAGGLFNCLGHYTWSDQNYHHGHNTGDPSGDGRSNGSAEEATAGKFGLQDVYFAGPTMTFQEPTFIPRQGAAEGEGYLIALLNHLDELRNDVVIFEARNLGKGPLAVIHLPLKLKLGLHGNWVDSREIEAWRRRRAENGDVGPLRVAKEPLPWQKKFAAAAQNGSNGV

SEQ ID NO: 4 - protein, 600 aa, synthetic construct
MAHIHDLAPEVSNYSSGRLTPPTPVRFPRTPVFASMNKPCRFEGDVFDLEVSGAIPPDIDGTFFRVQPDHRFPPLFEDDIHYNGDGSVTAIRISGGHADLRQRYVRTERYLLETRARRSLFGRYRNPWTDNESVRGVIRTASNTNVVFWRGALLAMKEDGPPFAMDPVTLETLGRYDFEGQILSPTFTAHPKIDPDTGEMVCFAYEAGGDGSDCSVDVAVWTVDADGKKVEECWYKAPFAGMIHDCGITKNWVVLPLTPIKMDLERMKRGGNKFAWDPSEDQWYGVVPRRGAKSDDIIWFRADNGFHGHVAGCYELPSGEIVFDLTVADGNXXXFFPPDDNITPPADGVAKRNRLSSPTVRWIFDPKAKKSAIRTEAAGDADIWVADERVKPALTWPTNGEFSRIDDRYVTKPYRHFWQAVVDPTRPYDFEKCGPPAGGLFNCLGHYTWSDQNYHHGHNTGDPSGDGRSNGSAEEATAGKFGLQDVYFAGPTMTFQEPTFIPRQGAAEGEGYLIALLNHLDELRNDVVIFEARNLGKGPLAVIHLPLKLKLGLHGNWVDSREIEAWRRRRAENGDVGPLRVAKEPLPWQKKFAAAAQNGS

SEQ ID NO: 5 - DNA, 1812 bp, Thermothelomyces thermophila
  source 1..1812: mol_type = genomic DNA
atggctcacatccacgacctggcgccggaagtaagcaactactcttctggtcgcctgaccccgccgaccccagttaggttcccgcgcaccccagtgttcgcatctatgaacaaaccgtgccgcttcgaaggtgacgttttcgacctggaagtttctggtgctatcccgccggacatcgacggtaccttcttccgcgttcagccggaccaccgcttcccgccgctgttcgaagacgacatccacttcaacggtgacggttctgttaccgctatccgcatctctggtggtcacgctgacctgcgccagcgctacgttcgcaccgaacgctacctgctggaaacccgcgctcgccgctctctgttcggtcgctaccgcaacccgtggaccgacaacgaatctgttcgcggtgttatccgcaccgcttctaacaccaacgttgttttctggcgcggtgctctgctggctatgaaagaagacggtccgccgttcgctatggacccggttaccctggaaaccctgggtcgctacgacttcgaaggtcagatcctgtctccgaccttcaccgctcacccgaaaatcgacccggacaccggtgaaatggtttgcttcgcttacgaagctggtggtgacggttctgactgctctgttgacgttgctgtttggaccgttgacgctgacggtaaaaaagttgaagaatgctggtacaaagctccgttcgctggtatgatccacgactgcggtatcaccaaaaactgggttgttctgccgctgaccccgatcaaaatggacctggaacgcatgaaacgcggtggtaacaaattcgcttgggacccgtctgaagaccagtggtacggtgttgttccgcgccgcggtgctaaatctgacgacatcatctggttccgcgctgacaacggcttccacggtcacgttgctggttgctacgaactgccgtctggtgaaatcgttttcgacctgacagttgcggacggcaacgtcttcttcttcttcccgccggacgacaacatcaccccgccggctgacggtgttgctaaacgcaaccgcctgtcttctccgaccgttcgctggatcttcgacccgaaagctaaaaaatctgctatccgcaccgaagctgctggtgacgctgacatctgggttgctgacgaacgcgttaaaccggctctgacctggccgaccaacggtgaattctctcgcatcgacgaccgctacgttaccaaaccgtaccgccacttctggcaggctgttgttgacccgacccgcccgtacgacttcgaaaaatgcggtccgccggctggtggtctgttcaactgcctgggtcactacacctggtctgaccagaactaccaccacggtcacaacaccggtgacccgtctggtgacggtcgctctaacggttctgctgaagaagctaccgctggtaaattcggcctgcaggacgtatacttcgccggtccgaccatgaccttccaggaaccgaccttcatcccgcgccagggtgctgctgaaggtgaaggttacctgatcgctctgctgaaccacctggacgaactgcgcaacgacgttgttatcttcgaagctcgcaacctgggtaaaggtccgctggctgttatccacctgccgctgaaactgaaactgggtctgcacggtaactgggttgactctcgcgaaatcgaagcttggcgccgccgccgcgctgaaaacggtgacgttggtccgctgcgcgttgctaaagaaccgctgccgtggcagaaaaaattcgctgctgctgctcagaacggttctaacggtgtttaa

SEQ ID NO: 6 - DNA, 30 bp, synthetic construct
  source 1..30: mol_type = other DNA
cgcggatccgatggctcacatccacgacct

SEQ ID NO: 7 - DNA, 35 bp, synthetic construct
  source 1..35: mol_type = other DNA
ataagaatgcggccgcttaaacaccgttagaaccg

SEQ ID NO: 8 - DNA, 1812 bp, synthetic construct
  source 1..1812: mol_type = other DNA
atggctcacatccacgacctggcgccggaagtaagcaactactcttctggtcgcctgaccccgccgaccccagttaggttcccgcgcaccccagtgttcgcatctatgaacaaaccgtgccgcttcgaaggtgacgttttcgacctggaagtttctggtgctatcccgccggacatcgacggtaccttcttccgcgttcagccggaccaccgcttcccgccgctgttcgaagacgacatccactataacggtgacggttctgttaccgctatccgcatctctggtggtcacgctgacctgcgccagcgctacgttcgcaccgaacgctacctgctggaaacccgcgctcgccgctctctgttcggtcgctaccgcaacccgtggaccgacaacgaatctgttcgcggtgttatccgcaccgcttctaacaccaacgttgttttctggcgcggtgctctgctggctatgaaagaagacggtccgccgttcgctatggacccggttaccctggaaaccctgggtcgctacgacttcgaaggtcagatcctgtctccgaccttcaccgctcacccgaaaatcgacccggacaccggtgaaatggtttgcttcgcttacgaagctggtggtgacggttctgactgctctgttgacgttgctgtttggaccgttgacgctgacggtaaaaaagttgaagaatgctggtacaaagctccgttcgctggtatgatccacgactgcggtatcaccaaaaactgggttgttctgccgctgaccccgatcaaaatggacctggaacgcatgaaacgcggtggtaacaaattcgcttgggacccgtctgaagaccagtggtacggtgttgttccgcgccgcggtgctaaatctgacgacatcatctggttccgcgctgacaacggcttccacggtcacgttgctggttgctacgaactgccgtctggtgaaatcgttttcgacctgacagttgcggacggcaacgtcttcttcttcttcccgccggacgacaacatcaccccgccggctgacggtgttgctaaacgcaaccgcctgtcttctccgaccgttcgctggatcttcgacccgaaagctaaaaaatctgctatccgcaccgaagctgctggtgacgctgacatctgggttgctgacgaacgcgttaaaccggctctgacctggccgaccaacggtgaattctctcgcatcgacgaccgctacgttaccaaaccgtaccgccacttctggcaggctgttgttgacccgacccgcccgtacgacttcgaaaaatgcggtccgccggctggtggtctgttcaactgcctgggtcactacacctggtctgaccagaactaccaccacggtcacaacaccggtgacccgtctggtgacggtcgctctaacggttctgctgaagaagctaccgctggtaaattcggcctgcaggacgtatacttcgccggtccgaccatgaccttccaggaaccgaccttcatcccgcgccagggtgctgctgaaggtgaaggttacctgatcgctctgctgaaccacctggacgaactgcgcaacgacgttgttatcttcgaagctcgcaacctgggtaaaggtccgctggctgttatccacctgccgctgaaactgaaactgggtctgcacggtaactgggttgactctcgcgaaatcgaagcttggcgccgccgccgcgctgaaaacggtgacgttggtccgctgcgcgttgctaaagaaccgctgccgtggcagaaaaaattcgctgctgctgctcagaacggttctaacggtgtttaa

SEQ ID NO: 9 - DNA, 28 bp, synthetic construct
  source 1..28: mol_type = other DNA
tataacggtgacggttctgttaccgcta

SEQ ID NO: 10 - DNA, 25 bp, synthetic construct
  source 1..25: mol_type = other DNA
gtggatgtcgtcttcgaacagcggc

SEQ ID NO: 11 - DNA, 1500 bp, synthetic construct
  source 1..1500: mol_type = other DNA
atggctcacatccacgacctggcgccggaagtaagcaactactcttctggtcgcctgaccccgccgaccccagttaggttcccgcgcaccccagtgttcgcatctatgaacaaaccgtgccgcttcgaaggtgacgttttcgacctggaagtttctggtgctatcccgccggacatcgacggtaccttcttccgcgttcagccggaccaccgcttcccgccgctgttcgaagacgacatccactggaacggtgacggttctgttaccgctatccgcatctctggtggtcacgctgacctgcgccagcgctacgttcgcaccgaacgctacctgctggaaacccgcgctcgccgctctctgttcggtcgctaccgcaacccgtggaccgacaacgaatctgttcgcggtgttatccgcaccgcttctaacaccaacgttgttttctggcgcggtgctctgctggctatgaaagaagacggtccgccgttcgctatggacccggttaccctggaaaccctgggtcgctacgacttcgaaggtcagatcctgtctccgaccttcaccgctcacccgaaaatcgacccggacaccggtgaaatggtttgcttcgcttacgaagctggtggtgacggttctgactgctctgttgacgttgctgtttggaccgttgacgctgacggtaaaaaagttgaagaatgctggtacaaagctccgttcgctggtatgatccacgactgcggtatcaccaaaaactgggttgttctgccgctgaccccgatcaaaatggacctggaacgcatgaaacgcggtggtaacaaattcgcttgggacccgtctgaagaccagtggtacggtgttgttccgcgccgcggtgctaaatctgacgacatcatctggttccgcgctgacaacggcttccacggtcacgttgctggttgctacgaactgccgtctggtgaaatcgttttcgacctgacagttgcggacggcaacgtcttcttcttcttcccgccggacgacaacatcaccccgccggctgacggtgttgctaaacgcaaccgcctgtcttctccgaccgttcgctggatcttcgacccgaaagctaaaaaatctgctatccgcaccgaagctgctggtgacgctgacatctgggttgctgacgaacgcgttaaaccggctctgacctggccgaccaacggtgaattctctcgcatcgacgaccgctacgttaccaaaccgtaccgccacttctggcaggctgttgttgacccgacccgcccgtacgacttcgaaaaatgcggtccgccggctggtggtctgttcaactgcctgggtcactacacctggtctgaccagaactaccaccacggtcacaacaccggtgacccgtctggtgacggtcgctctaacggttctgctgaagaagctaccgctggtaaattcggcctgcaggacgtatacttcgccggtccgaccatgaccttccaggaaccgaccttc

SEQ ID NO: 12 - DNA, 28 bp, synthetic construct
  source 1..28: mol_type = other DNA
tggaacggtgacggttctgttaccgcta

SEQ ID NO: 13 - DNA, 25 bp, synthetic construct
  source 1..25: mol_type = other DNA
gtggatgtcgtcttcgaacagcggc

SEQ ID NO: 14 - DNA, 1812 bp, synthetic construct
  source 1..1812: mol_type = other DNA
atggctcacatccacgacctggcgccggaagtaagcaactactcttctggtcgcctgaccccgccgaccccagttaggttcccgcgcaccccagtgttcgcatctatgaacaaaccgtgccgcttcgaaggtgacgttttcgacctggaagtttctggtgctatcccgccggacatcgacggtaccttcttccgcgttcagccggaccaccgcttcccgccgctgttcgaagacgacatccactataacggtgacggttctgttaccgctatccgcatctctggtggtcacgctgacctgcgccagcgctacgttcgcaccgaacgctacctgctggaaacccgcgctcgccgctctctgttcggtcgctaccgcaacccgtggaccgacaacgaatctgttcgcggtgttatccgcaccgcttctaacaccaacgttgttttctggcgcggtgctctgctggctatgaaagaagacggtccgccgttcgctatggacccggttaccctggaaaccctgggtcgctacgacttcgaaggtcagatcctgtctccgaccttcaccgctcacccgaaaatcgacccggacaccggtgaaatggtttgcttcgcttacgaagctggtggtgacggttctgactgctctgttgacgttgctgtttggaccgttgacgctgacggtaaaaaagttgaagaatgctggtacaaagctccgttcgctggtatgatccacgactgcggtatcaccaaaaactgggttgttctgccgctgaccccgatcaaaatggacctggaacgcatgaaacgcggtggtaacaaattcgcttgggacccgtctgaagaccagtggtacggtgttgttccgcgccgcggtgctaaatctgacgacatcatctggttccgcgctgacaacggcttccacggtcacgttgctggttgctacgaactgccgtctggtgaaatcgttttcgacctgacagttgcggacggcaacnnknnknnkttcttcccgccggacgacaacatcaccccgccggctgacggtgttgctaaacgcaaccgcctgtcttctccgaccgttcgctggatcttcgacccgaaagctaaaaaatctgctatccgcaccgaagctgctggtgacgctgacatctgggttgctgacgaacgcgttaaaccggctctgacctggccgaccaacggtgaattctctcgcatcgacgaccgctacgttaccaaaccgtaccgccacttctggcaggctgttgttgacccgacccgcccgtacgacttcgaaaaatgcggtccgccggctggtggtctgttcaactgcctgggtcactacacctggtctgaccagaactaccaccacggtcacaacaccggtgacccgtctggtgacggtcgctctaacggttctgctgaagaagctaccgctggtaaattcggcctgcaggacgtatacttcgccggtccgaccatgaccttccaggaaccgaccttcatcccgcgccagggtgctgctgaaggtgaaggttacctgatcgctctgctgaaccacctggacgaactgcgcaacgacgttgttatcttcgaagctcgcaacctgggtaaaggtccgctggctgttatccacctgccgctgaaactgaaactgggtctgcacggtaactgggttgactctcgcgaaatcgaagcttggcgccgccgccgcgctgaaaacggtgacgttggtccgctgcgcgttgctaaagaaccgctgccgtggcagaaaaaattcgctgctgctgctcagaacggttctaacggtgtttaa

SEQ ID NO: 15 - DNA, 37 bp, synthetic construct
  source 1..37: mol_type = other DNA
aacnnknnknnkttcttcccgccggacgacaacatca

SEQ ID NO: 16 - DNA, 25 bp, synthetic construct
  source 1..25: mol_type = other DNA
gccgtccgcaactgtcaggtcgaaa